European Patent Application EP 4 759 926 A1, published June 17, 2026. Title: Pluripotent stem cells with doubled chromosomes. Applicant: Tokyo Metropolitan Institute of Medical Science. The sequence listing filed with the application follows.

SEQUENCE LISTING (6 sequences)

SEQ ID NO: 1 - DNA, 23 bp, synthetic construct
  source 1..23: mol_type = other DNA
ccctcatgttcatacacctatcc

SEQ ID NO: 2 - DNA, 21 bp, synthetic construct
  source 1..21: mol_type = other DNA
agcctctgttgtcagattcac

SEQ ID NO: 3 - DNA, 26 bp, synthetic construct
  source 1..26: mol_type = other DNA
cccattctcctcctatccctcaaccc

SEQ ID NO: 4 - DNA, 18 bp, synthetic construct
  source 1..18: mol_type = other DNA
gatttggacctgcgagcg

SEQ ID NO: 5 - DNA, 18 bp, synthetic construct
  source 1..18: mol_type = other DNA
gcggctgtctccacaagt

SEQ ID NO: 6 - DNA, 16 bp, synthetic construct
  source 1..16: mol_type = other DNA
ctgacctgaaggctct